European Patent Specification EP 3 529 274 B1, published April 17, 2024. Title: A MONOCLONAL ANTIBODY AND A METHOD OF USE FOR THE TREATMENT OF SYSTEMIC LUPUS ERYTHEMATOSUS. Applicant: Biocon Limited. The sequence listing filed with the application follows.

SEQUENCE LISTING (5 sequences)

SEQ ID NO: 1 - protein, 119 aa, Artificial Sequence
  Synthetic Construct
EVQLVESGGGLVKPGGSLKLSCAASGFKFSRYAMSWVRQAPGKRLEWVATISSGGSYIYYPDSVKGRFTISRDNVKNTLYLQMSSLRSEDTAMYYCARRDYDLDYFDSWGQGTLVTVSS

SEQ ID NO: 2 - protein, 107 aa, Artificial Sequence
  Synthetic Construct
DIQMTQSPSSLSASVGDRVTITCKASRDIRSYLTWYQQKPGKAPKTLIYYATSLADGVPSRFSGSGSGQDYSLTISSLESDDTATYYCLQHGESPFTLGSGTKLEIK

SEQ ID NO: 3 - DNA, 357 bp, Artificial Sequence
  Synthetic construct
  exon (1)..(357)
gaagtgcagctggtggagtctgggggaggcttagtgaagcctggagggtccctgaaactctcctgtgcagcctctggattcaagtttagtagatatgccatgtcttgggttcgccaggctccggggaagaggctggagtgggtcgcaaccattagtagtggtggtagttacatctactatccagacagtgtgaagggtcgattcaccatctccagagacaatgtcaagaacaccctgtatctgcaaatgagcagtctgaggtctgaggacacggccatgtattactgtgcaagacgagattacgacctggactactttgactcctggggccaaggcacccttgtcaccgtctcctca

SEQ ID NO: 4 - DNA, 318 bp, Artificial Sequence
  Synthetic Construct
  exon (1)..(318)
gacatccagatgacccagtctccatcctccctgtctgcatcggtgggagacagagtcactatcacttgcaaggcgagtcgggacattagaagctatttaacctggtaccagcagaaaccagggaaagctcctaagaccctgatctattatgcaacaagcttggcagatggggtcccgtcgagattcagtggcagtggatctgggcaagattattctctcaccatcagcagcctggagtctgacgatacagcaacttactactgtctacaacatggtgagagtccaacgctcggctcggggaccaagctggaaatcaaa

SEQ ID NO: 5 - protein, 109 aa, Artificial Sequence
  Synthetic Construct
DIQMTQSPSSLSASVGDRVTITCKASRDIRSYLTWYQQKPGKAPKTLIYYATSLADGVPSRFSGSGSGQDYSLTISSLESDDTATYYCLQHGESPFTFGSGTKLEIKRA